European Patent Application EP 4 202 043 A1, published June 28, 2023. Title: A METHOD FOR GENETIC MODIFICATION FOR HIGH CG CONTENT MICROORGANISMS. Applicant: Technische Universitaet Muenchen. The sequence listing filed with the application follows.

SEQUENCE LISTING (27 sequences)

SEQ ID NO: 1 - protein, 1379 aa, Artificial Sequence
  Cas9 protein sequence with Nuclear localization sequence (NLS)
MDKKYSIGLDIGTNSVGWAVITDEYKVPSKKFKVLGNTDRHSIKKNLIGALLFDSGETAEATRLKRTARRRYTRRKNRICYLQEIFSNEMAKVDDSFFHRLEESFLVEEDKKHERHPIFGNIVDEVAYHEKYPTIYHLRKKLVDSTDKADLRLIYLALAHMIKFRGHFLIEGDLNPDNSDVDKLFIQLVQTYNQLFEENPINASGVDAKAILSARLSKSRRLENLIAQLPGEKKNGLFGNLIALSLGLTPNFKSNFDLAEDAKLQLSKDTYDDDLDNLLAQIGDQYADLFLAAKNLSDAILLSDILRVNTEITKAPLSASMIKRYDEHHQDLTLLKALVRQQLPEKYKEIFFDQSKNGYAGYIDGGASQEEFYKFIKPILEKMDGTEELLVKLNREDLLRKQRTFDNGSIPHQIHLGELHAILRRQEDFYPFLKDNREKIEKILTFRIPYYVGPLARGNSRFAWMTRKSEETITPWNFEEVVDKGASAQSFIERMTNFDKNLPNEKVLPKHSLLYEYFTVYNELTKVKYVTEGMRKPAFLSGEQKKAIVDLLFKTNRKVTVKQLKEDYFKKIECFDSVEISGVEDRFNASLGTYHDLLKIIKDKDFLDNEENEDILEDIVLTLTLFEDREMIEERLKTYAHLFDDKVMKQLKRRRYTGWGRLSRKLINGIRDKQSGKTILDFLKSDGFANRNFMQLIHDDSLTFKEDIQKAQVSGQGDSLHEHIANLAGSPAIKKGILQTVKVVDELVKVMGRHKPENIVIEMARENQTTQKGQKNSRERMKRIEEGIKELGSQILKEHPVENTQLQNEKLYLYYLQNGRDMYVDQELDINRLSDYDVDHIVPQSFLKDDSIDNKVLTRSDKNRGKSDNVPSEEVVKKMKNYWRQLLNAKLITQRKFDNLTKAERGGLSELDKAGFIKRQLVETRQITKHVAQILDSRMNTKYDENDKLIREVKVITLKSKLVSDFRKDFQFYKVREINNYHHAHDAYLNAVVGTALIKKYPKLESEFVYGDYKVYDVRKMIAKSEQEIGKATAKYFFYSNIMNFFKTEITLANGEIRKRPLIETNGETGEIVWDKGRDFATVRKVLSMPQVNIVKKTEVQTGGFSKESILPKRNSDKLIARKKDWDPKKYGGFDSPTVAYSVLVVAKVEKGKSKKLKSVKELLGITIMERSSFEKNPIDFLEAKGYKEVKKDLIIKLPKYSLFELENGRKRMLASAGELQKGNELALPSKYVNFLYLASHYEKLKGSPEDNEQKQLFVEQHKHYLDEIIEQISEFSKRVILADANLDKVLSAYNKHRDKPIREQAENIIHLFTLTNLGAPAAFKYFDTTIDRKRYTSTKEVLDATLIHQSITGLYETRIDLSQLGGDSRADPKKKRKV

SEQ ID NO: 2 - protein, 1368 aa, Artificial Sequence [sequence omitted]

SEQ ID NO: 3 - RNA, 4140 nt, Artificial Sequence
  Cas9 mRNA sequence with NLS
auggacaagaaguacucgaucggccucgacaucggcaccaacucggucggcugggccgucaucaccgacgaguacaagguccccucgaagaaguucaagguccucggcaacaccgaccgccacucgaucaagaagaaccucaucggcgcccuccucuucgacucgggcgagaccgccgaggccacccgccucaagcgcaccgcccgccgccgcuacacccgccgcaagaaccgcaucugcuaccuccaggagaucuucucgaacgagauggccaaggucgacgacucguucuuccaccgccucgaggagucguuccucgucgaggaggacaagaagcacgagcgccaccccaucuucggcaacaucgucgacgaggucgccuaccacgagaaguaccccaccaucuaccaccuccgcaagaagcucgucgacucgaccgacaaggccgaccuccgccucaucuaccucgcccucgcccacaugaucaaguuccgcggccacuuccucaucgagggcgaccucaaccccgacaacucggacgucgacaagcucuucauccagcucguccagaccuacaaccagcucuucgaggagaaccccaucaacgccucgggcgucgacgccaaggccauccucucggcccgccucucgaagucgcgccgccucgagaaccucaucgcccagcuccccggcgagaagaagaacggccucuucggcaaccucaucgcccucucgcucggccucacccccaacuucaagucgaacuucgaccucgccgaggacgccaagcuccagcucucgaaggacaccuacgacgacgaccucgacaaccuccucgcccagaucggcgaccaguacgccgaccucuuccucgccgccaagaaccucucggacgccauccuccucucggacauccuccgcgucaacaccgagaucaccaaggccccccucucggccucgaugaucaagcgcuacgacgagcaccaccaggaccucacccuccucaaggcccucguccgccagcagcuccccgagaaguacaaggagaucuucuucgaccagucgaagaacggcuacgccggcuacaucgacggcggcgccucgcaggaggaguucuacaaguucaucaagcccauccucgagaagauggacggcaccgaggagcuccucgucaagcucaaccgcgaggaccuccuccgcaagcagcgcaccuucgacaacggcucgaucccccaccagauccaccucggcgagcuccacgccauccuccgccgccaggaggacuucuaccccuuccucaaggacaaccgcgagaagaucgagaagauccucaccuuccgcauccccuacuacgucggcccccucgcccgcggcaacucgcgcuucgccuggaugacccgcaagucggaggagaccaucacccccuggaacuucgaggaggucgucgacaagggcgccucggcccagucguucaucgagcgcaugaccaacuucgacaagaaccuccccaacgagaagguccuccccaagcacucgcuccucuacgaguacuucaccgucuacaacgagcucaccaaggucaaguacgucaccgagggcaugcgcaagcccgccuuccucucgggcgagcagaagaaggccaucgucgaccuccucuucaagaccaaccgcaaggucaccgucaagcagcucaaggaggacuacuucaagaagaucgagugcuucgacucggucgagaucucgggcgucgaggaccgcuucaacgccucgcucggcaccuaccacgaccuccucaagaucaucaaggacaaggacuuccucgacaacgaggagaacgaggacauccucgaggacaucguccucacccucacccucuucgaggaccgcgagaugaucgaggagcgccucaagaccuacgcccaccucuucgacgacaaggucaugaagcagcucaagcgccgccgcuacaccggcuggggccgccucucgcgcaagcucaucaacggcauccgcgacaagcagucgggcaagaccauccucgacuuccucaagucggacggcuucgccaaccgcaacuucaugcagcucauccacgacgacucgcucaccuucaaggaggacauccagaaggcccaggucucgggccagggcgacucgcuccacgagcacaucgccaaccucgccggcucgcccgccaucaagaagggcauccuccagaccgucaaggucgucgacgagcucgucaaggucaugggccgccacaagcccgagaacaucgucaucgagauggcccgcgagaaccagaccacccagaagggccagaagaacucgcgcgagcgcaugaagcgcaucgaggagggcaucaaggagcucggcucgcagauccucaaggagcaccccgucgagaacacccagcuccagaacgagaagcucuaccucuacuaccuccagaacggccgcgacauguacgucgaccaggagcucgacaucaaccgccucucggacuacgacgucgaccacaucgucccccagucguuccucaaggacgacucgaucgacaacaagguccucacccgcucggacaagaaccgcggcaagucggacaacguccccucggaggaggucgucaagaagaugaagaacuacuggcgccagcuccucaacgccaagcucaucacccagcgcaaguucgacaaccucaccaaggccgagcgcggcggccucucggagcucgacaaggccggcuucaucaagcgccagcucgucgagacccgccagaucaccaagcacgucgcccagauccucgacucgcgcaugaacaccaaguacgacgagaacgacaagcucauccgcgaggucaaggucaucacccucaagucgaagcucgucucggacuuccgcaaggacuuccaguucuacaagguccgcgagaucaacaacuaccaccacgcccacgacgccuaccucaacgccgucgucggcaccgcccucaucaagaaguaccccaagcucgagucggaguucgucuacggcgacuacaaggucuacgacguccgcaagaugaucgccaagucggagcaggagaucggcaaggccaccgccaaguacuucuucuacucgaacaucaugaacuucuucaagaccgagaucacccucgccaacggcgagauccgcaagcgcccccucaucgagaccaacggcgagaccggcgagaucgucugggacaagggccgcgacuucgccaccguccgcaagguccucucgaugccccaggucaacaucgucaagaagaccgagguccagaccggcggcuucucgaaggagucgauccuccccaagcgcaacucggacaagcucaucgcccgcaagaaggacugggaccccaagaaguacggcggcuucgacucgcccaccgucgccuacucgguccucgucgucgccaaggucgagaagggcaagucgaagaagcucaagucggucaaggagcuccucggcaucaccaucauggagcgcucgucguucgagaagaaccccaucgacuuccucgaggccaagggcuacaaggaggucaagaaggaccucaucaucaagcuccccaaguacucgcucuucgagcucgagaacggccgcaagcgcaugcucgccucggccggcgagcuccagaagggcaacgagcucgcccuccccucgaaguacgucaacuuccucuaccucgccucgcacuacgagaagcucaagggcucgcccgaggacaacgagcagaagcagcucuucgucgagcagcacaagcacuaccucgacgagaucaucgagcagaucucggaguucucgaagcgcgucauccucgccgacgccaaccucgacaagguccucucggccuacaacaagcaccgcgacaagcccauccgcgagcaggccgagaacaucauccaccucuucacccucaccaaccucggcgcccccgccgccuucaaguacuucgacaccaccaucgaccgcaagcgcuacaccucgaccaaggagguccucgacgccacccucauccaccagucgaucaccggccucuacgagacccgcaucgaccucucgcagcucggcggcgacucgcgcgccgaccccaagaagaagcgcaaggucuag

SEQ ID NO: 4 - RNA, 4119 nt, Artificial Sequence
  Cas9 mRNA sequence without NLS
auggacaagaaguacucgaucggccucgacaucggcaccaacucggucggcugggccgucaucaccgacgaguacaagguccccucgaagaaguucaagguccucggcaacaccgaccgccacucgaucaagaagaaccucaucggcgcccuccucuucgacucgggcgagaccgccgaggccacccgccucaagcgcaccgcccgccgccgcuacacccgccgcaagaaccgcaucugcuaccuccaggagaucuucucgaacgagauggccaaggucgacgacucguucuuccaccgccucgaggagucguuccucgucgaggaggacaagaagcacgagcgccaccccaucuucggcaacaucgucgacgaggucgccuaccacgagaaguaccccaccaucuaccaccuccgcaagaagcucgucgacucgaccgacaaggccgaccuccgccucaucuaccucgcccucgcccacaugaucaaguuccgcggccacuuccucaucgagggcgaccucaaccccgacaacucggacgucgacaagcucuucauccagcucguccagaccuacaaccagcucuucgaggagaaccccaucaacgccucgggcgucgacgccaaggccauccucucggcccgccucucgaagucgcgccgccucgagaaccucaucgcccagcuccccggcgagaagaagaacggccucuucggcaaccucaucgcccucucgcucggccucacccccaacuucaagucgaacuucgaccucgccgaggacgccaagcuccagcucucgaaggacaccuacgacgacgaccucgacaaccuccucgcccagaucggcgaccaguacgccgaccucuuccucgccgccaagaaccucucggacgccauccuccucucggacauccuccgcgucaacaccgagaucaccaaggccccccucucggccucgaugaucaagcgcuacgacgagcaccaccaggaccucacccuccucaaggcccucguccgccagcagcuccccgagaaguacaaggagaucuucuucgaccagucgaagaacggcuacgccggcuacaucgacggcggcgccucgcaggaggaguucuacaaguucaucaagcccauccucgagaagauggacggcaccgaggagcuccucgucaagcucaaccgcgaggaccuccuccgcaagcagcgcaccuucgacaacggcucgaucccccaccagauccaccucggcgagcuccacgccauccuccgccgccaggaggacuucuaccccuuccucaaggacaaccgcgagaagaucgagaagauccucaccuuccgcauccccuacuacgucggcccccucgcccgcggcaacucgcgcuucgccuggaugacccgcaagucggaggagaccaucacccccuggaacuucgaggaggucgucgacaagggcgccucggcccagucguucaucgagcgcaugaccaacuucgacaagaaccuccccaacgagaagguccuccccaagcacucgcuccucuacgaguacuucaccgucuacaacgagcucaccaaggucaaguacgucaccgagggcaugcgcaagcccgccuuccucucgggcgagcagaagaaggccaucgucgaccuccucuucaagaccaaccgcaaggucaccgucaagcagcucaaggaggacuacuucaagaagaucgagugcuucgacucggucgagaucucgggcgucgaggaccgcuucaacgccucgcucggcaccuaccacgaccuccucaagaucaucaaggacaaggacuuccucgacaacgaggagaacgaggacauccucgaggacaucguccucacccucacccucuucgaggaccgcgagaugaucgaggagcgccucaagaccuacgcccaccucuucgacgacaaggucaugaagcagcucaagcgccgccgcuacaccggcuggggccgccucucgcgcaagcucaucaacggcauccgcgacaagcagucgggcaagaccauccucgacuuccucaagucggacggcuucgccaaccgcaacuucaugcagcucauccacgacgacucgcucaccuucaaggaggacauccagaaggcccaggucucgggccagggcgacucgcuccacgagcacaucgccaaccucgccggcucgcccgccaucaagaagggcauccuccagaccgucaaggucgucgacgagcucgucaaggucaugggccgccacaagcccgagaacaucgucaucgagauggcccgcgagaaccagaccacccagaagggccagaagaacucgcgcgagcgcaugaagcgcaucgaggagggcaucaaggagcucggcucgcagauccucaaggagcaccccgucgagaacacccagcuccagaacgagaagcucuaccucuacuaccuccagaacggccgcgacauguacgucgaccaggagcucgacaucaaccgccucucggacuacgacgucgaccacaucgucccccagucguuccucaaggacgacucgaucgacaacaagguccucacccgcucggacaagaaccgcggcaagucggacaacguccccucggaggaggucgucaagaagaugaagaacuacuggcgccagcuccucaacgccaagcucaucacccagcgcaaguucgacaaccucaccaaggccgagcgcggcggccucucggagcucgacaaggccggcuucaucaagcgccagcucgucgagacccgccagaucaccaagcacgucgcccagauccucgacucgcgcaugaacaccaaguacgacgagaacgacaagcucauccgcgaggucaaggucaucacccucaagucgaagcucgucucggacuuccgcaaggacuuccaguucuacaagguccgcgagaucaacaacuaccaccacgcccacgacgccuaccucaacgccgucgucggcaccgcccucaucaagaaguaccccaagcucgagucggaguucgucuacggcgacuacaaggucuacgacguccgcaagaugaucgccaagucggagcaggagaucggcaaggccaccgccaaguacuucuucuacucgaacaucaugaacuucuucaagaccgagaucacccucgccaacggcgagauccgcaagcgcccccucaucgagaccaacggcgagaccggcgagaucgucugggacaagggccgcgacuucgccaccguccgcaagguccucucgaugccccaggucaacaucgucaagaagaccgagguccagaccggcggcuucucgaaggagucgauccuccccaagcgcaacucggacaagcucaucgcccgcaagaaggacugggaccccaagaaguacggcggcuucgacucgcccaccgucgccuacucgguccucgucgucgccaaggucgagaagggcaagucgaagaagcucaagucggucaaggagcuccucggcaucaccaucauggagcgcucgucguucgagaagaaccccaucgacuuccucgaggccaagggcuacaaggaggucaagaaggaccucaucaucaagcuccccaaguacucgcucuucgagcucgagaacggccgcaagcgcaugcucgccucggccggcgagcuccagaagggcaacgagcucgcccuccccucgaaguacgucaacuuccucuaccucgccucgcacuacgagaagcucaagggcucgcccgaggacaacgagcagaagcagcucuucgucgagcagcacaagcacuaccucgacgagaucaucgagcagaucucggaguucucgaagcgcgucauccucgccgacgccaaccucgacaagguccucucggccuacaacaagcaccgcgacaagcccauccgcgagcaggccgagaacaucauccaccucuucacccucaccaaccucggcgcccccgccgccuucaaguacuucgacaccaccaucgaccgcaagcgcuacaccucgaccaaggagguccucgacgccacccucauccaccagucgaucaccggccucuacgagacccgcaucgaccucucgcagcucggcggcgacucgcgcgccgacuag

SEQ ID NO: 5 - RNA, 76 nt, Artificial Sequence
  trans-activating crispr RNA (tracrRNA)
guuuuagagcuagaaauagcaaguuaaaauaaggcuaguccguuaucaacuugaaaaaguggcaccgagucggugc

SEQ ID NO: 6 - DNA, 3712 bp, Artificial Sequence
  Donor DNA including a knock in gene of interest (a new promoter for D9 desaturase gene), selection marker (ura 5 gene -Orotate phosphoribosyltransferase-), and homology arms
gaagaccagaggccgtgggaagaatagtgcgcggggtagacgtaatagtgcgtacccgtagacattacgcagaggctgtatcggtggagagacgatgagctggtggtcctggtggatgatgaccagtagtggagataatgatcatggccgggtatacgaccctcaggcacaagattgtcagatacgtggagcgttcaggcaccatcgctcatcatcggagcgagacacgtgggattgtgcaatcagcttccgcgacccacgccatgtccatggacgatcgtgacgacgcgaggccatctccgctccgtgcgccgctgctccattgctgcatcgctccacccctggccatcgtcacggtcacggacaccggccggtgccggtgggccatggcgccgggtcagacgctatggggcacgtgctggagctacgccggccatgacaaggcggaatggcgcagacgcagtcggcgctgtggcggcggccggcttgggccaatccacgcagcgccgttgcagcgtccatctgacgctggagtggatgggggcggggcccacgatatggtgtggtggcgtaccccgcagcagctgggcgatggaattggcatggaggaggaagcatcttatcttgtggtgatggattgccgccccagaggcgggcgtcgggcgtcgggcggaggcatgaggcatattacagtacaagaggcgatgaaatctgataaaccgagcggggaggggtgtgggggtcggcgcgggcgcccacgccgggtcgtggtgatgtgatgatgaagatggtgaccgtatgaccgtcgctggaaggatgccgaagatttgtcgatggggagggggatatgcgccgcgacaccgccgctgcggtcgcccaatgtgcgccctgtccatcgccgcttatgtcctgtgccgtcgctgtcgatgtcgaagggggtgctcggcgtgaggactcactgagttgtcggacgagaaacagaaggacccacgccgctgtagtcgacacacccagcggaggcagactgtccaggaccaccatggctgtgaaccctgagctcgaggtcgtcggcgttaaagttgaggccgatcatgacagctcaactttcacgatttatcggggtcaaatgtatcatcccacgtcagctctggttggtgcctgattcaacccatctccgccggatagcgggccgagacgcaatccgcacttgagctcgttcatctctcctgcattactcacaatggctgctaccgacttcaaggccaactttattgagacggcgatcaacaccggggtcctcctcttcggcgagttcaccctcaagtctggccggtgagtaggtgcgacctgccgccgtcgtcgaatgtccaggctgacggccagcaagtccccgtacttcttcaacgccgggctcctgtacgacggcgctcttctctccgcgaccgccgacgcgtttgccggcacgctttccgcgatccccgagttcgatgtcctcttcggccccgcgtacaagggcatccccctcgcggccgtcacctgcgtcgctctcgcgaacaagggcatcaacaaggtctactgctacaaccgcaaggagaagaaggaccacggcgagggcggcacgctcgtcggcgcgcccatggcggacaagaaggtcgtgatcatcgacgacgttatgacggccggcacggcgattcgcgaagccatcgccattcttaaggagcagccgggcgcacagctcgttggtatcgtgcagctcgtcgaccgccaggagcgcggcaagggctcgacctcgaccagccaggaggtcgctgccgagtttggcgttccagttcttcccatcatctccatcggggacattatcacgtacctcaaggcccgtgggggatacgaggagcaggtcaaggctatcgaggcgtaccgcgccgagtacggcgttgtcgcctgaggcagctggtgtccgaggcgtcgaagccaagcgcggccgggatgtgaattgagcgggagataggatcccccatggtgccagatcttgggtaattgcgcgctgaaggccagattagagcatctcatcatgtactttatacaatgcattgcgcgtctcttggggtggagcagtaagcgttgtagatggtcgtcacaatcatagaggcgccctgcgcgtcccgcatgccgagtttgtaaaggtctctctcggtcgcatatgaacagctcaatccgctgcataaccaggaggcatgagaggggctggactactcatcgtcggggcagaagcgctgcgtgtccggacgaacttccggcatgtaggtggaccacacttcgggtgaaggggtgcgcctctgtgcgtatgagatgggacgcgcgcactttgcgagtttagagctttggacacttagacgacatgtcgaaggctctaaacgtacatccaccaacacagctaacagagggagtaagcggggctggactctcctcgttattatgagccgagaccccggcccggcggcagctcacggcagtcaggggcgtcggtagatgcccgggtgattcgacgtcaccacatttgggactatcaacacgacctcgtcagtgacagatgctggtgccccttccgacctcattatgcatggtagcgagggcgggacgaacgagcagtgctcgagcagcacatgtgcacattctcgctcgataaaaaagtgcaagtctgtcggcgtcatcccgacacgctcgcgacgaatgtccgcgtgtgtggtgtgctgctattccccgaaaacgccccgagggcaacatccgttcacccgcgctcacccagagcccacctgttctcacgccagccccaggccgcaggctgtataaagctcttccccgtccacttatctttcctcccattcttctctcccagtccaaacacaatgtcggcctccacaaagcaggctgcgaccaccgtcgctcagccatcgggcaagcccgtcaccaacgtgattgaccccgagcgcgacgactttatcgttcccgacaactacgtcacccgcacagtcgagaacatgaagatgctcccccccgtcacatggcgcaacctccacaagaacattcagtggatttccttccttgccctcaccatcccccccgcaatggccatctacggcctttgcaccgtcccagtccagacaaagacttttatctggtctgtcgtctactacttcatcactggtctcggcatcaccgccggctaccaccgtctttgggcccaccgctcctacaacgcttcaaagccactccagtacttcctcgcccttgctggcgcaggctcggtccagggctcgatcagatggtggtcccgcggccaccgcgcccaccaccgctacaccgacaccaaactcgacccctactcggctcacgagggcttctggcacgctcacatgggctggatgctcatcaagcctcgcggcaagatcggtgtcgctgacatttccgacctgagcaagaaccccgtcgtcaagtggcagcacaacaactacgtcgccctcctcttcttcatgggtctcgctttccccactcttgtcgctggtctcggctggggagactggtggggcggcctcttcttcgccggtgccgctcgcctcgtctttgtccaccactcgaccttttgcgtcaactcgcttgcccactggctcggtgagaccccctttgacaacaagcacacccccaaggagtcttc

SEQ ID NO: 7 - DNA, 3825 bp, Artificial Sequence
  Donor DNA including a knock in gene of interest (a new promoter for D9 desaturase gene), selection marker (ura 5 gene Orotate phosphoribosyltransferase), and homology arms
gaagaccagaggccgtgggaagaatagtgcgcggggtagacgtaatagtgcgtacccgtagacattacgcagaggctgtatcggtggagagacgatgagctggtggtcctggtggatgatgaccagtagtggagataatgatcatggccgggtatacgaccctcaggcacaagattgtcagatacgtggagcgttcaggcaccatcgctcatcatcggagcgagacacgtgggattgtgcaatcagcttccgcgacccacgccatgtccatggacgatcgtgacgacgcgaggccatctccgctccgtgcgccgctgctccattgctgcatcgctccacccctggccatcgtcacggtcacggacaccggccggtgccggtgggccatggcgccgggtcagacgctatggggcacgtgctggagctacgccggccatgacaaggcggaatggcgcagacgcagtcggcgctgtggcggcggccggcttgggccaatccacgcagcgccgttgcagcgtccatctgacgctggagtggatgggggcggggcccacgatatggtgtggtggcgtaccccgcagcagctgggcgatggaattggcatggaggaggaagcatcttatcttgtggtgatggattgccgccccagaggcgggcgtcgggcgtcgggcggaggcatgaggcatattacagtacaagaggcgatgaaatctgataaaccgagcggggaggggtgtgggggtcggcgcgggcgcccacgccgggtcgtggtgatgtgatgatgaagatggtgaccgtatgaccgtcgctggaaggatgccgaagatttgtcgatggggagggggatatgcgccgcgacaccgccgctgcggtcgcccaatgtgcgccctgtccatcgccgcttatgtcctgtgccgtcgctgtcgatgtcgaagggggtgctcggcgtgaggactcactgagttgtcggacgagaaacagaaggacccacgccgctgtagtcgacacacccagcggaggcagactgtccaggaccaccatggctgtgaaccctgagctcgaggtcgtcggcgttaaagttgaggccgatcatgacagctcaactttcacgatttatcggggtcaaatgtatcatcccacgtcagctctggttggtgcctgattcaacccatctccgccggatagcgggccgagacgcaatccgcacttgagctcgttcatctctcctgcattactcacaatggctgctaccgacttcaaggccaactttattgagacggcgatcaacaccggggtcctcctcttcggcgagttcaccctcaagtctggccggtgagtaggtgcgacctgccgccgtcgtcgaatgtccaggctgacggccagcaagtccccgtacttcttcaacgccgggctcctgtacgacggcgctcttctctccgcgaccgccgacgcgtttgccggcacgctttccgcgatccccgagttcgatgtcctcttcggccccgcgtacaagggcatccccctcgcggccgtcacctgcgtcgctctcgcgaacaagggcatcaacaaggtctactgctacaaccgcaaggagaagaaggaccacggcgagggcggcacgctcgtcggcgcgcccatggcggacaagaaggtcgtgatcatcgacgacgttatgacggccggcacggcgattcgcgaagccatcgccattcttaaggagcagccgggcgcacagctcgttggtatcgtgcagctcgtcgaccgccaggagcgcggcaagggctcgacctcgaccagccaggaggtcgctgccgagtttggcgttccagttcttcccatcatctccatcggggacattatcacgtacctcaaggcccgtgggggatacgaggagcaggtcaaggctatcgaggcgtaccgcgccgagtacggcgttgtcgcctgaggcagctggtgtccgaggcgtcgaagccaagcgcggccgggatgtgaattgagcgggagataggatcccccatggtgccagatcttgggtaattgcgcgctgaaggccagattagagcatctcatcatgtactttatacaatgcattgcgcgtctcttgggtcacccaggaaaaattttgtggcggcgcctgggcggggcatggaccgggcggaagattgcaactggcgagctgctcggcagggtccgctcataccgctcgctcagctccctctctccttccttccttctttccttcccctcctgccctcctggcatcaaattaacgtgaggggatcggataaacattgcgccaaatcaccccgtacggtgagcaagccgacgtcaggctgccacacaagggccctctagcggcgttatagaccccgccacacgtcataacaccataacgccgtgactgggctttgagtagacaaaggcaattcagggtctgttggaggggcgagctccagtgccagcgcactgtaaaatccgcgtgcgatccgctttctctcttcactcccaccctctctctctcctccaaaaaacagtgagtagcaccaacgacaaccatggcaatggtggtcgccaaagaggcaaagacagcgagcgcactgcgaccgacaacgacctgcccgtcatcgactcgaacaacctgcagcaccatcgctctcgtcatcgccgcgcgccacttgccctgcactccttccccccacccctcatccatcccatcctttcctctcgaccatgcaaggccacctgcctcgagtgcatgcgctcttggcgatgctcgcgcattggtatcgtggtcgtctgcatcgtcgtcaaacagacggagcacgacgaccgtgacgaattggatggcacaaagggtccatgtcaaatttgacctcccgcttccaccttcaaccttcctccatccaacatcctccgcctttgactcgcaatgcgcatgctgtctttgtctccccactcccaccattgactgccactctcagagaatgtcgactaacattgcagacaaaacctattcaaaatgtcggcctccacaaagcaggctgcgaccaccgtcgctcagccatcgggcaagcccgtcaccaacgtgattgaccccgagcgcgacgactttatcgttcccgacaactacgtcacccgcacagtcgagaacatgaagatgctcccccccgtcacatggcgcaacctccacaagaacattcagtggatttccttccttgccctcaccatcccccccgcaatggccatctacggcctttgcaccgtcccagtccagacaaagacttttatctggtctgtcgtctactacttcatcactggtctcggcatcaccgccggctaccaccgtctttgggcccaccgctcctacaacgcttcaaagccactccagtacttcctcgcccttgctggcgcaggctcggtccagggctcgatcagatggtggtcccgcggccaccgcgcccaccaccgctacaccgacaccaaactcgacccctactcggctcacgagggcttctggcacgctcacatgggctggatgctcatcaagcctcgcggcaagatcggtgtcgctgacatttccgacctgagcaagaaccccgtcgtcaagtggcagcacaacaactacgtcgccctcctcttcttcatgggtctcgctttccccactcttgtcgctggtctcggctggggagactggtggggcggcctcttcttcgccggtgccgctcgcctcgtctttgtccaccactcgaccttttgcgtcaactcgcttgcccactggctcggtgagaccccctttgacaacaagcacacccccaaggagtcttc

SEQ ID NO: 8 - DNA, 3698 bp, Artificial Sequence
  Donor DNA including a knock in gene of interest (a new promoter for D12 desaturase gene), selection marker (ura 5 gene -Orotate phosphoribosyltransferase-), and homology arms
cctgtacccgaccacactgacctttgcatacgcgatgcgcggcgtgattatggcgctggagatacacgcgacgtcattcaagctctggcgcctcccaccgccccgcgagcccgtgtggaatctcctcctgcgttccgtcgacgacacgctgcgccgcctaaaagggggcggggggcaggtggcggcgcgcatcgcgatcgcatctgtcggcgccgcgcgagagacgatccggcggtggcgcgccgagctggtccgccgcccattcaatcccaatcacgcgccgcggcccacaatcacccccgacggcccgagccccgcgaccgcgaaagccgtcgctgccaagacgggggtcgcgggggtggtccccggcacgctgtcggcgggtttgttcagcggcttcgagcccgcggccgggttcgagctgcagggatttgatcctatggtcacgtcgtttgcggagtggattgctggtatcgactggaaccagtttgtggtgacggagtaggggggggggggggggggggggggggggggggggggggcgggggcatcaacttgatgatgattatgggcggctgcagggttgcagcacacacttgcatcctcttctacactgcatatgtatatgcatgacttggtgaacgactatcgagaatcttgcgaatgacaagcgtattccaccacccgacttgttatgcagtgcaagtaagcccgactcgtcatcggatagcctcgggtcatgctcgacacggtgaccgggtatcatcattgatcatggatcatgggtcatggagtcatcgctggaaggatgccgaagatttgtcgatggggagggggatatgcgccgcgacaccgccgctgcggtcgcccaatgtgcgccctgtccatcgccgcttatgtcctgtgccgtcgctgtcgatgtcgaagggggtgctcggcgtgaggactcactgagttgtcggacgagaaacagaaggacccacgccgctgtagtcgacacacccagcggaggcagactgtccaggaccaccatggctgtgaaccctgagctcgaggtcgtcggcgttaaagttgaggccgatcatgacagctcaactttcacgatttatcggggtcaaatgtatcatcccacgtcagctctggttggtgcctgattcaacccatctccgccggatagcgggccgagacgcaatccgcacttgagctcgttcatctctcctgcattactcacaatggctgctaccgacttcaaggccaactttattgagacggcgatcaacaccggggtcctcctcttcggcgagttcaccctcaagtctggccggtgagtaggtgcgacctgccgccgtcgtcgaatgtccaggctgacggccagcaagtccccgtacttcttcaacgccgggctcctgtacgacggcgctcttctctccgcgaccgccgacgcgtttgccggcacgctttccgcgatccccgagttcgatgtcctcttcggccccgcgtacaagggcatccccctcgcggccgtcacctgcgtcgctctcgcgaacaagggcatcaacaaggtctactgctacaaccgcaaggagaagaaggaccacggcgagggcggcacgctcgtcggcgcgcccatggcggacaagaaggtcgtgatcatcgacgacgttatgacggccggcacggcgattcgcgaagccatcgccattcttaaggagcagccgggcgcacagctcgttggtatcgtgcagctcgtcgaccgccaggagcgcggcaagggctcgacctcgaccagccaggaggtcgctgccgagtttggcgttccagttcttcccatcatctccatcggggacattatcacgtacctcaaggcccgtgggggatacgaggagcaggtcaaggctatcgaggcgtaccgcgccgagtacggcgttgtcgcctgaggcagctggtgtccgaggcgtcgaagccaagcgcggccgggatgtgaattgagcgggagataggatcccccatggtgccagatcttgggtaattgcgcgctgaaggccagattagagcatctcatcatgtactttatacaatgcattgcgcgtctcttggggtggagcagtaagcgttgtagatggtcgtcacaatcatagaggcgccctgcgcgtcccgcatgccgagtttgtaaaggtctctctcggtcgcatatgaacagctcaatccgctgcataaccaggaggcatgagaggggctggactactcatcgtcggggcagaagcgctgcgtgtccggacgaacttccggcatgtaggtggaccacacttcgggtgaaggggtgcgcctctgtgcgtatgagatgggacgcgcgcactttgcgagtttagagctttggacacttagacgacatgtcgaaggctctaaacgtacatccaccaacacagctaacagagggagtaagcggggctggactctcctcgttattatgagccgagaccccggcccggcggcagctcacggcagtcaggggcgtcggtagatgcccgggtgattcgacgtcaccacatttgggactatcaacacgacctcgtcagtgacagatgctggtgccccttccgacctcattatgcatggtagcgagggcgggacgaacgagcagtgctcgagcagcacatgtgcacattctcgctcgataaaaaagtgcaagtctgtcggcgtcatcccgacacgctcgcgacgaatgtccgcgtgtgtggtgtgctgctattccccgaaaacgccccgagggcaacatccgttcacccgcgctcacccagagcccacctgttctcacgccagccccaggccgcaggctgtataaagctcttccccgtccacttatctttcctcccattcttctctcccagtccaaacacaatgtctgccgccaccctgcgccagcgtaacgtcgacaagccaggtgctgccgacaaggccgagctcctccgtgaagccgaggacctcgagctcaccgagggccagaagtttgtcgtgcccaactttaccgtcaagcagctcttggacgccattccgtgagtgccctttgccccccccccatggcgcagaggcggatgtcggatggcttgcgtgagccacggcgtcggtggcaaacccatcactctaatcaatccgataagggacgcctgatggcggtgctcctcgcgtgccaactacggtgggccgcgggccgtcatggtgacgacgagacggacacaggacctcgttttgcgattccgtccgattaaactttacacccagaaccacgctcaccccagcgcccactgctacaagcgctcggcgttcaagtcgtcgctttacgtcctccaggactttgtcctcctcgccgccctcgtctacggcgcctaccacattgactccttcttgagccgcttgtgagtatttcccatcagatatcggtggagggaccgggaatccagcgacgcgggggtcgagtggagccatcatgtggctttttcatcccacctcgccgtgcctgcgtgccaagacaaggcaaccgtaggcacaatcgttgctccaccaccccaagtccccctcatggcagcatcatgctcggacttgctctcatgggtctctgatgcatgctcctgcggccagccgctaacatcgcagcaaccttggctcggttgcccacaccgccgccaagatcggcctctggt

SEQ ID NO: 9 - DNA, 3811 bp, Artificial Sequence
  Donor DNA including a knock in gene of interest (a new promoter for D12 desaturase gene), selection marker (ura 5 gene -Orotate phosphoribosyltransferase-), and homology arms
cctgtacccgaccacactgacctttgcatacgcgatgcgcggcgtgattatggcgctggagatacacgcgacgtcattcaagctctggcgcctcccaccgccccgcgagcccgtgtggaatctcctcctgcgttccgtcgacgacacgctgcgccgcctaaaagggggcggggggcaggtggcggcgcgcatcgcgatcgcatctgtcggcgccgcgcgagagacgatccggcggtggcgcgccgagctggtccgccgcccattcaatcccaatcacgcgccgcggcccacaatcacccccgacggcccgagccccgcgaccgcgaaagccgtcgctgccaagacgggggtcgcgggggtggtccccggcacgctgtcggcgggtttgttcagcggcttcgagcccgcggccgggttcgagctgcagggatttgatcctatggtcacgtcgtttgcggagtggattgctggtatcgactggaaccagtttgtggtgacggagtaggggggggggggggggggggggggggggggggggggggcgggggcatcaacttgatgatgattatgggcggctgcagggttgcagcacacacttgcatcctcttctacactgcatatgtatatgcatgacttggtgaacgactatcgagaatcttgcgaatgacaagcgtattccaccacccgacttgttatgcagtgcaagtaagcccgactcgtcatcggatagcctcgggtcatgctcgacacggtgaccgggtatcatcattgatcatggatcatgggtcatggagtcatcgctggaaggatgccgaagatttgtcgatggggagggggatatgcgccgcgacaccgccgctgcggtcgcccaatgtgcgccctgtccatcgccgcttatgtcctgtgccgtcgctgtcgatgtcgaagggggtgctcggcgtgaggactcactgagttgtcggacgagaaacagaaggacccacgccgctgtagtcgacacacccagcggaggcagactgtccaggaccaccatggctgtgaaccctgagctcgaggtcgtcggcgttaaagttgaggccgatcatgacagctcaactttcacgatttatcggggtcaaatgtatcatcccacgtcagctctggttggtgcctgattcaacccatctccgccggatagcgggccgagacgcaatccgcacttgagctcgttcatctctcctgcattactcacaatggctgctaccgacttcaaggccaactttattgagacggcgatcaacaccggggtcctcctcttcggcgagttcaccctcaagtctggccggtgagtaggtgcgacctgccgccgtcgtcgaatgtccaggctgacggccagcaagtccccgtacttcttcaacgccgggctcctgtacgacggcgctcttctctccgcgaccgccgacgcgtttgccggcacgctttccgcgatccccgagttcgatgtcctcttcggccccgcgtacaagggcatccccctcgcggccgtcacctgcgtcgctctcgcgaacaagggcatcaacaaggtctactgctacaaccgcaaggagaagaaggaccacggcgagggcggcacgctcgtcggcgcgcccatggcggacaagaaggtcgtgatcatcgacgacgttatgacggccggcacggcgattcgcgaagccatcgccattcttaaggagcagccgggcgcacagctcgttggtatcgtgcagctcgtcgaccgccaggagcgcggcaagggctcgacctcgaccagccaggaggtcgctgccgagtttggcgttccagttcttcccatcatctccatcggggacattatcacgtacctcaaggcccgtgggggatacgaggagcaggtcaaggctatcgaggcgtaccgcgccgagtacggcgttgtcgcctgaggcagctggtgtccgaggcgtcgaagccaagcgcggccgggatgtgaattgagcgggagataggatcccccatggtgccagatcttgggtaattgcgcgctgaaggccagattagagcatctcatcatgtactttatacaatgcattgcgcgtctcttgggtcacccaggaaaaattttgtggcggcgcctgggcggggcatggaccgggcggaagattgcaactggcgagctgctcggcagggtccgctcataccgctcgctcagctccctctctccttccttccttctttccttcccctcctgccctcctggcatcaaattaacgtgaggggatcggataaacattgcgccaaatcaccccgtacggtgagcaagccgacgtcaggctgccacacaagggccctctagcggcgttatagaccccgccacacgtcataacaccataacgccgtgactgggctttgagtagacaaaggcaattcagggtctgttggaggggcgagctccagtgccagcgcactgtaaaatccgcgtgcgatccgctttctctcttcactcccaccctctctctctcctccaaaaaacagtgagtagcaccaacgacaaccatggcaatggtggtcgccaaagaggcaaagacagcgagcgcactgcgaccgacaacgacctgcccgtcatcgactcgaacaacctgcagcaccatcgctctcgtcatcgccgcgcgccacttgccctgcactccttccccccacccctcatccatcccatcctttcctctcgaccatgcaaggccacctgcctcgagtgcatgcgctcttggcgatgctcgcgcattggtatcgtggtcgtctgcatcgtcgtcaaacagacggagcacgacgaccgtgacgaattggatggcacaaagggtccatgtcaaatttgacctcccgcttccaccttcaaccttcctccatccaacatcctccgcctttgactcgcaatgcgcatgctgtctttgtctccccactcccaccattgactgccactctcagagaatgtcgactaacattgcagacaaaacctattcaaaatgtctgccgccaccctgcgccagcgtaacgtcgacaagccaggtgctgccgacaaggccgagctcctccgtgaagccgaggacctcgagctcaccgagggccagaagtttgtcgtgcccaactttaccgtcaagcagctcttggacgccattccgtgagtgccctttgccccccccccatggcgcagaggcggatgtcggatggcttgcgtgagccacggcgtcggtggcaaacccatcactctaatcaatccgataagggacgcctgatggcggtgctcctcgcgtgccaactacggtgggccgcgggccgtcatggtgacgacgagacggacacaggacctcgttttgcgattccgtccgattaaactttacacccagaaccacgctcaccccagcgcccactgctacaagcgctcggcgttcaagtcgtcgctttacgtcctccaggactttgtcctcctcgccgccctcgtctacggcgcctaccacattgactccttcttgagccgcttgtgagtatttcccatcagatatcggtggagggaccgggaatccagcgacgcgggggtcgagtggagccatcatgtggctttttcatcccacctcgccgtgcctgcgtgccaagacaaggcaaccgtaggcacaatcgttgctccaccaccccaagtccccctcatggcagcatcatgctcggacttgctctcatgggtctctgatgcatgctcctgcggccagccgctaacatcgcagcaaccttggctcggttgcccacaccgccgccaagatcggcctctggt

SEQ ID NO: 10 - DNA, 4601 bp, Artificial Sequence
  Donor DNA including a knock in gene of interest (Elongase coding sequence, aldo keto reductase promoter and terminator), selection marker (ura 5 gene -Orotate phosphoribosyltransferase-), and homology arms
gaagacaacagcaatcagacgcgtcttgcgggtgatggcctcggagccccaagcaaagttgcccgagtccagacggagggcgcggtacttggtgttgccgccacgggtgcgcacagtgtggatacgcttcgaagtgtcgagcttggtcatggccgactgacggccgagctcgaacttgcgcttcttgcggctgcctgtcagtatattgcaacgggaacatcgagttggtgcagggcagtaatgggacaagtgcgcagatttccctccctccgcttgcttgccggcagagcttcttctcccgaatccatcacaccgttccccgaatctgcacacttgaccccctgctagcccgcacaggcaagccactcactagtgggcgcggcgagcgccggatgcactgcgcttgtggcgggagtcacgagagatacccatttctgtcgttagtactaaaacgtgtgacaagtgccggagcacctccaggacaaggacagcggggcagacaggcttcgcggatggacaggatgcaggcgcagtcgccgaaagttcgtctggcgcatgtatttgccaagcgccgtcgaatgctgcagcggagtggtcgctggaaggatgccgaagatttgtcgatggggagggggatatgcgccgcgacaccgccgctgcggtcgcccaatgtgcgccctgtccatcgccgcttatgtcctgtgccgtcgctgtcgatgtcgaagggggtgctcggcgtgaggactcactgagttgtcggacgagaaacagaaggacccacgccgctgtagtcgacacaccttcgttaggcagactgtccaggaccaccatggctgtgaaccctgagctcgaggtcgtcggcgttaaagttgaggccgatcatgacagctcaactttcacgatttatcggggtcaaatgtatcatcccacgtcagctctggttggtgcctgattcaacccatctccgccggatagcgggccgagacgcaatccgcacttgagctcgttcatctctcctgcattactcacaatggctgctaccgacttcaaggccaactttattgagacggcgatcaacaccggggtcctcctcttcggcgagttcaccctcaagtctggccggtgagtaggtgcgacctgccgccgtcgtcgaatgtccaggctgacggccagcaagtccccgtacttcttcaacgccgggctcctgtacgacggcgctcttctctccgcgaccgccgacgcgtttgccggcacgctttccgcgatccccgagttcgatgtcctcttcggccccgcgtacaagggcatccccctcgcggccgtcacctgcgtcgctctcgcgaacaagggcatcaacaaggtctactgctacaaccgcaaggagaagaaggaccacggcgagggcggcacgctcgtcggcgcgcccatggcggacaagaaggtcgtgatcatcgacgacgttatgacggccggcacggcgattcgcgaagccatcgccattcttaaggagcagccgggcgcacagctcgttggtatcgtgcagctcgtcgaccgccaggagcgcggcaagggctcgacctcgaccagccaggaggtcgctgccgagtttggcgttccagttcttcccatcatctccatcggggacattatcacgtacctcaaggcccgtgggggatacgaggagcaggtcaaggctatcgaggcgtaccgcgccgagtacggcgttgtcgcctgaggcagctggtgtccgaggcgtcgaagccaagcgcggccgggatgtgaattgagcgggagataggatcccccatggtgccagatcttgggtaattgcgcgctgaaggccagattagagcatctcatcatgtactttatacaatgcattgcgcgtctcttggggtggagcagtaagcgttgtagatggtcgtcacaatcatagaggcgccctgcgcgtcccgcatgccgagtttgtaaaggtctctctcggtcgcatatgaacagctcaatccgctgcataaccaggaggcatgagaggggctggactactcatcgtcggggcagaagcgctgcgtgtccggacgaacttccggcatgtaggtggaccacacttcgggtgaaggggtgcgcctctgtgcgtatgagatgggacgcgcgcactttgcgagtttagagctttggacacttagacgacatgtcgaaggctctaaacgtacatccaccaacacagctaacagagggagtaagcggggctggactctcctcgttattatgagccgagaccccggcccggcggcagctcacggcagtcaggggcgtcggtagatgcccgggtgattcgacgtcaccacatttgggactatcaacacgacctcgtcagtgacagatgctggtgccccttccgacctcattatgcatggtagcgagggcgggacgaacgagcagtgctcgagcagcacatgtgcacattctcgctcgataaaaaagtgcaagtctgtcggcgtcatcccgacacgctcgcgacgaatgtccgcgtgtgtggtgtgctgctattccccgaaaacgccccgagggcaacatccgttcacccgcgctcacccagagcccacctgttctcacgccagccccaggccgcaggctgtataaagctcttccccgtccacttatctttcctcccattcttctctcccagtccaaacacaatggagtcgggccctatgcctgccggcatccccttccccgagtactacgactttttcatggactggaagactcccctcgccattgccgctacctacaccgttgccgtcggccttttcaaccccaaggtcggtaaggtctcgcgcgttgtcgccaagtcagccaacgccaagccagccgagcgtacccagtcgggcgccgcgatgaccgctttcgtcttcgtccacaacctcatcctttgcgtctactcgggcattaccttctaccacatgtttccagccatggttaagaacttccgtactcacaccctccacgaggcttactgcgacaccgaccaatcgctctggaataacgccctcggctactggggctacctcttctacctctcaaagttctacgaggtcatcgacaccattatcattatcctcaagggccgtcgctcgtcccttctccagacctaccaccacgccggcgctatgatcaccatgtggtcgggcatcaactaccaagccaccccaatctggatcttcgttgtcttcaactcgttcatccacaccattatgtactgctactacgccttcacctcgattggcttccacccacccggcaagaagtacctcacctcgatgcaaatcacccagtttctcgttggcatcaccatcgccgtttcgtacctcttcgtcccaggctgcatccgtacccccggcgcccagatggcggtctggatcaacgtcggttacctcttccccctcacctacctcttcgtcgactttgctaagcgcacctactcgaagcgcaccgcgatcgcggctcagaagaaggcccagtaggcgccggtggttgtagcagtatatgcatcgttaatgggattgatcgtccgcggctatcgtcgaggttgtccaccgccgccctcagcttatcactcgctcgcttcatgtatgtgtatggcaactgtacggcaaagattgaagtgtcgagttccttttagtatcagatgtgacaaagtagagacgtcgagagcatctctgggccgcagcagcaagctcatctctcagtctccttcatgtcacgttatacattgccatctacagccaccttattattagagcatctcatcatgtactttatacaatgcattgcgcgtctcttgggtcaatgttcactttacaatgtcgtgacgtcgcacgcggtcgcctcctcctctcgcgtcagtacttctttcccttgcccttcccccagcgttcggcaacaaggacgcgcgaagcgccaactactgcctcgacgaggtcgcgcacgtcattagcggtgaccggaacaccatactgggccgacaaatggttggcaacggcagctagtggctcagggcgagccaacgcgaacaccgcaacctcgaaaacacgagccgcgtccgccgccggaatgtcgatgagcgcgcttccgcccacctgtgtcaaggtggggatgaacgtcgcccaccacactgcccgaagagcgtcctgtccgccctcagaacgaggaagggccttgatcgtagttaaaacgagtgtgtagctcgtttgtaagatccgggcaacgtggggtcgggctggcgtcggcccatctcgcatcagccgcgcaggaacatttactcaccgagtgcggcctccagagttgtgctctgatcgaaaatggcgtgcaagacgccgccaatgcctcccgcacgatcgccaacaatccgtttgacctcagctaaggtgaagtcaaggtgcattcccagggcggccgggaacgcaacaggtccgttggtcatcgtgcggtttaagtccgcggcgcgtcggacgatcgggcgataagagagcggcgtgcaatatcgcgtagcctcagacgcggccggcgtcagagagacacgcgaggttgcgcgcgtcttc

SEQ ID NO: 11 - DNA, 5914 bp, Artificial Sequence
  Donor DNA including a knock in gene of interest (oleate hydratase coding sequence, transcription elongation factor 2 promoter and terminator), selection marker (ura 5 gene -Orotate phosphoribosyltransferase-), and homology arms
gaagacaacagcaatcagacgcgtcttgcgggtgatggcctcggagccccaagcaaagttgcccgagtccagacggagggcgcggtacttggtgttgccgccacgggtgcgcacagtgtggatacgcttcgaagtgtcgagcttggtcatggccgactgacggccgagctcgaacttgcgcttcttgcggctgcctgtcagtatattgcaacgggaacatcgagttggtgcagggcagtaatgggacaagtgcgcagatttccctccctccgcttgcttgccggcagagcttcttctcccgaatccatcacaccgttccccgaatctgcacacttgaccccctgctagcccgcacaggcaagccactcactagtgggcgcggcgagcgccggatgcactgcgcttgtggcgggagtcacgagagatacccatttctgtcgttagtactaaaacgtgtgacaagtgccggagcacctccaggacaaggacagcggggcagacaggcttcgcggatggacaggatgcaggcgcagtcgccgaaagttcgtctggcgcatgtatttgccaagcgccgtcgaatgctgcagcggagtggtcgctggaaggatgccgaagatttgtcgatggggagggggatatgcgccgcgacaccgccgctgcggtcgcccaatgtgcgccctgtccatcgccgcttatgtcctgtgccgtcgctgtcgatgtcgaagggggtgctcggcgtgaggactcactgagttgtcggacgagaaacagaaggacccacgccgctgtagtcgacacaccttcgttaggcagactgtccaggaccaccatggctgtgaaccctgagctcgaggtcgtcggcgttaaagttgaggccgatcatgacagctcaactttcacgatttatcggggtcaaatgtatcatcccacgtcagctctggttggtgcctgattcaacccatctccgccggatagcgggccgagacgcaatccgcacttgagctcgttcatctctcctgcattactcacaatggctgctaccgacttcaaggccaactttattgagacggcgatcaacaccggggtcctcctcttcggcgagttcaccctcaagtctggccggtgagtaggtgcgacctgccgccgtcgtcgaatgtccaggctgacggccagcaagtccccgtacttcttcaacgccgggctcctgtacgacggcgctcttctctccgcgaccgccgacgcgtttgccggcacgctttccgcgatccccgagttcgatgtcctcttcggccccgcgtacaagggcatccccctcgcggccgtcacctgcgtcgctctcgcgaacaagggcatcaacaaggtctactgctacaaccgcaaggagaagaaggaccacggcgagggcggcacgctcgtcggcgcgcccatggcggacaagaaggtcgtgatcatcgacgacgttatgacggccggcacggcgattcgcgaagccatcgccattcttaaggagcagccgggcgcacagctcgttggtatcgtgcagctcgtcgaccgccaggagcgcggcaagggctcgacctcgaccagccaggaggtcgctgccgagtttggcgttccagttcttcccatcatctccatcggggacattatcacgtacctcaaggcccgtgggggatacgaggagcaggtcaaggctatcgaggcgtaccgcgccgagtacggcgttgtcgcctgaggcagctggtgtccgaggcgtcgaagccaagcgcggccgggatgtgaattgagcgggagataggatcccccatggtgccagatcttgggtaattgcgcgctgaaggccagattagagcatctcatcatgtactttatacaatgcattgcgcgtctcttgggtcacccaggaaaaattttgtggcggcgcctgggcggggcatggaccgggcggaagattgcaactggcgagctgctcggcagggtccgctcataccgctcgctcagctccctctctccttccttccttctttccttcccctcctgccctcctggcatcaaattaacgtgaggggatcggataaacattgcgccaaatcaccccgtacggtgagcaagccgacgtcaggctgccacacaagggccctctagcggcgttatagaccccgccacacgtcataacaccataacgccgtgactgggctttgagtagacaaaggcaattcagggtctgttggaggggcgagctccagtgccagcgcactgtaaaatccgcgtgcgatccgctttctctcttcactcccaccctctctctctcctccaaaaaacagtgagtagcaccaacgacaaccatggcaatggtggtcgccaaagaggcaaagacagcgagcgcactgcgaccgacaacgacctgcccgtcatcgactcgaacaacctgcagcaccatcgctctcgtcatcgccgcgcgccacttgccctgcactccttccccccacccctcatccatcccatcctttcctctcgaccatgcaaggccacctgcctcgagtgcatgcgctcttggcgatgctcgcgcattggtatcgtggtcgtctgcatcgtcgtcaaacagacggagcacgacgaccgtgacgaattggatggcacaaagggtccatgtcaaatttgacctcccgcttccaccttcaaccttcctccatccaacatcctccgcctttgactcgcaatgcgcatgctgtctttgtctccccactcccaccattgactgccactctcagagaatgtcgactaacattgcagacaaaacctattcaaaatgtcctcgaacctctcgcacaaggcctacatgatcggcgccggcatcggcaacctttcggcggccgtttacctcatccgtgacggcgagtggaacggcgaggacattaccatcatgggccttgacatgcacggcgctaacgacggtgagtcggctgccaccttccaacaccagtacggtcaccgtgagctcggcaacgacgccggctttattaacaggggtggccgtatgcttaacgaggagacctacgagaacctctgggacgtcctctcggccgtcccgtcccttgacaaccccggcaagtcggtcaccgacgacattctcgacttcgaccacgcgcaccctacccacgacgttgcccgcctcattgaccgtgacggcatccgcaacaagggcgagaacgactacaagcacatgcagttcgacaacaaggaccgctaccttctcaccaagctcatgaccatgcccgagtcggacgaggccaagctcgacgacatctcgatcgagcagtggttcgaggagacccctcactttttcactaccaacttttggtacatgtgggagactaccttcgccttcaagcgcgtctcatcggctatggagctccgtcgctacatgaaccgcatgatcctcgagttctcacgtatccaaacccttgccggcgttaccaggtcgccttacaaccaatacgagtcgatcattctcccaatgcgtaccttcctcgagggcaagggcgtcaagttcgtcaatgagctcaagatcaccgagtttgtctttaaggacacccctctccgtgacgagattatcgtcaccggcctcgactacgagaatgtccgcaccggcgagaagggcaggatcgacgtcgcggagggcgacttcgtcttcgacaccaacggctcgatcactgactcgtcatcgatcggcgacctcgacacccccatcgtcgaggacatgcgttacgcgccctcggcgcttctctggaagcaagccaccgagcacttctacgacctcggcaaccccgacaagttctttggcgaccgcgcgcagtcggagtggacctcgttcaccgtcactacctcctcgcacgagctcatcaatgagatctcgaggatcaccaagcagctccccggtaacgcgcttaacaccttcgtcgactcgaacgtccttctctcgatcgttgtccaccaccaaccccactaccacgcccagaaggagaacgagggcgtcttctggggctactgcctcttcccccgcaaggacggtgactacgtcaagaagcccttcatcgagatgaccggtcgtgagatgctcgaggagactctcggccacctcgaggccctcgacgagtcgggtaccctcgctgccaggcgccaagagatcatggactccgtcgttaactcgattccatcgcacatgccctacgcctcggctctcttcaaccgtcgcgccgtcggcgaccgccctctcgttgtccccaagcactcgaagaacctcgccttcatctcgcaattcgctgagctccccttcgacatggtcttcaccgagcaatactccgtccgctgcgctcaggttgccgtctacaagttccttggtatccccgaggacaagcttaccaagatgcaccactacgagaaggaccccaaggttctcgctaaggctgccgtcaccatgttccgttagttgtgcttcgagcgtgcttatttgtatgtctcttcatccttagttctcctcagataggcctctcggcgatgcaccgttgaaggctaccattctaaagtttcgttgcgggtgtgagtgttgagatagcgttgcttgacctgtagaatacgaggcagcaccaacgccgataacatccaagtcaggcttagcactggtcctgcttggttgctgatgaggcgcggggtcgacgagccgatctcgttgaagccgtgtatcgtatcagctttcgagtctactgtaggctttgttgtggtgtacgcccctttagctgcccactgcagatcgtagatgtcgcatgcatgttcgcgtcgactaccccaaacgtctgatatctgatgttcagtacatcgggggtcattttctctgtgcttcgatgatgccacgccgctgatctgctgaaggtagagagagagtacgagagatcccactagcagttctggccatgcattgtcgctgttgccagcagtcgagttctctggtgccgtttcaaacgatggatcgtgagcttgcatgcttggttgaatcagcccaatagctggcagtcaaatacattctgactccgctaattcgcctctgactaattagagcatctcatcatgtactttatacaatgcattgcgcgtctcttgggtcaatgttcactttacaatgtcgtgacgtcgcacgcggtcgcctcctcctctcgcgtcagtacttctttcccttgcccttcccccagcgttcggcaacaaggacgcgcgaagcgccaactactgcctcgacgaggtcgcgcacgtcattagcggtgaccggaacaccatactgggccgacaaatggttggcaacggcagctagtggctcagggcgagccaacgcgaacaccgcaacctcgaaaacacgagccgcgtccgccgccggaatgtcgatgagcgcgcttccgcccacctgtgtcaaggtggggatgaacgtcgcccaccacactgcccgaagagcgtcctgtccgccctcagaacgaggaagggccttgatcgtagttaaaacgagtgtgtagctcgtttgtaagatccgggcaacgtggggtcgggctggcgtcggcccatctcgcatcagccgcgcaggaacatttactcaccgagtgcggcctccagagttgtgctctgatcgaaaatggcgtgcaagacgccgccaatgcctcccgcacgatcgccaacaatccgtttgacctcagctaaggtgaagtcaaggtgcattcccagggcggccgggaacgcaacaggtccgttggtcatcgtgcggtttaagtccgcggcgcgtcggacgatcgggcgataagagagcggcgtgcaatatcgcgtagcctcagacgcggccggcgtcagagagacacgcgaggttgcgcgcgtcttc

SEQ ID NO: 12 - DNA, 5430 bp, Artificial Sequence
  Donor DNA including a knock in gene of interest (delta9 desaturase coding sequence, aldo keto reductase promoter and terminator), selection marker (ura 5 gene -Orotate phosphoribosyltransferase-), and homology arms
aacagcaatcagacgcgtcttgcgggtgatggcctcggagccccaagcaaagttgcccgagtccagacggagggcgcggtacttggtgttgccgccacgggtgcgcacagtgtggatacgcttcgaagtgtcgagcttggtcatggccgactgacggccgagctcgaacttgcgcttcttgcggctgcctgtcagtatattgcaacgggaacatcgagttggtgcagggcagtaatgggacaagtgcgcagatttccctccctccgcttgcttgccggcagagcttcttctcccgaatccatcacaccgttccccgaatctgcacacttgaccccctgctagcccgcacaggcaagccactcactagtgggcgcggcgagcgccggatgcactgcgcttgtggcgggagtcacgagagatacccatttctgtcgttagtactaaaacgtgtgacaagtgccggagcacctccaggacaaggacagcggggcagacaggcttcgcggatggacaggatgcaggcgcagtcgccgaaagttcgtctggcgcatgtatttgccaagcgccgtcgaatgctgcagcggagtggtcgctggaaggatgccgaagatttgtcgatggggagggggatatgcgccgcgacaccgccgctgcggtcgcccaatgtgcgccctgtccatcgccgcttatgtcctgtgccgtcgctgtcgatgtcgaagggggtgctcggcgtgaggactcactgagttgtcggacgagaaacagaaggacccacgccgctgtagtcgacacaccttcgttaggcagactgtccaggaccaccatggctgtgaaccctgagctcgaggtcgtcggcgttaaagttgaggccgatcatgacagctcaactttcacgatttatcggggtcaaatgtatcatcccacgtcagctctggttggtgcctgattcaacccatctccgccggatagcgggccgagacgcaatccgcacttgagctcgttcatctctcctgcattactcacaatggctgctaccgacttcaaggccaactttattgagacggcgatcaacaccggggtcctcctcttcggcgagttcaccctcaagtctggccggtgagtaggtgcgacctgccgccgtcgtcgaatgtccaggctgacggccagcaagtccccgtacttcttcaacgccgggctcctgtacgacggcgctcttctctccgcgaccgccgacgcgtttgccggcacgctttccgcgatccccgagttcgatgtcctcttcggccccgcgtacaagggcatccccctcgcggccgtcacctgcgtcgctctcgcgaacaagggcatcaacaaggtctactgctacaaccgcaaggagaagaaggaccacggcgagggcggcacgctcgtcggcgcgcccatggcggacaagaaggtcgtgatcatcgacgacgttatgacggccggcacggcgattcgcgaagccatcgccattcttaaggagcagccgggcgcacagctcgttggtatcgtgcagctcgtcgaccgccaggagcgcggcaagggctcgacctcgaccagccaggaggtcgctgccgagtttggcgttccagttcttcccatcatctccatcggggacattatcacgtacctcaaggcccgtgggggatacgaggagcaggtcaaggctatcgaggcgtaccgcgccgagtacggcgttgtcgcctgaggcagctggtgtccgaggcgtcgaagccaagcgcggccgggatgtgaattgagcgggagataggatcccccatggtgccagatcttgggtaattgcgcgctgaaggccagattagagcatctcatcatgtactttatacaatgcattgcgcgtctcttggggtggagcagtaagcgttgtagatggtcgtcacaatcatagaggcgccctgcgcgtcccgcatgccgagtttgtaaaggtctctctcggtcgcatatgaacagctcaatccgctgcataaccaggaggcatgagaggggctggactactcatcgtcggggcagaagcgctgcgtgtccggacgaacttccggcatgtaggtggaccacacttcgggtgaaggggtgcgcctctgtgcgtatgagatgggacgcgcgcactttgcgagtttagagctttggacacttagacgacatgtcgaaggctctaaacgtacatccaccaacacagctaacagagggagtaagcggggctggactctcctcgttattatgagccgagaccccggcccggcggcagctcacggcagtcaggggcgtcggtagatgcccgggtgattcgacgtcaccacatttgggactatcaacacgacctcgtcagtgacagatgctggtgccccttccgacctcattatgcatggtagcgagggcgggacgaacgagcagtgctcgagcagcacatgtgcacattctcgctcgataaaaaagtgcaagtctgtcggcgtcatcccgacacgctcgcgacgaatgtccgcgtgtgtggtgtgctgctattccccgaaaacgccccgagggcaacatccgttcacccgcgctcacccagagcccacctgttctcacgccagccccaggccgcaggctgtataaagctcttccccgtccacttatctttcctcccattcttctctcccagtccaaacacaatgtccgcttccacaaagcaggctgcgaccaccgtcgctcagccatcgggcaagcccgtcaccaacgtgattgaccccgagcgcgacgactttatcgttcccgacaactacgtcacccgcacagtcgagaacatgaagatgctcccccccgtcacatggcgcaacctccacaagaacattcagtggatttccttccttgccctcaccatcccccccgcaatggccatctacggcctttgcaccgtcccagtccagacaaagacttttatctggtctgtcgtctactacttcatcactggtctcggcatcaccgccggctaccaccgtctttgggcccaccgctcctacaacgcttcaaagccactccagtacttcctcgcccttgctggcgcaggctcggtccagggctcgatcagatggtggtcccgcggccaccgcgcccaccaccgctacaccgacaccaaactcgacccctactcggctcacgagggcttctggcacgctcacatgggctggatgctcatcaagcctcgcggcaagatcggtgtcgctgacatttccgacctgagcaagaaccccgtcgtcaagtggcagcacaacaactacgtcgccctcctcttcttcatgggtctcgctttccccactcttgtcgctggtctcggctggggagactggtggggcggcctcttcttcgccggtgccgctcgcctcgtctttgtccaccactcgaccttttgcgtcaactcgcttgcccactggctcggtgagaccccctttgacaacaagcacacccccaaggaccactttatcaccgcgcttgtcaccgtcggcgagggctaccacaacttccaccaccagttccccatggacttccgcaacgccatcaagtggtaccagtacgaccccacaaagtggttcatctggaccatggctcagctcggcctcgcctcgcacctcaaaaagttccccgacaacgagatcaagaagggccagtacaccatgaagctcatgcagcttcaggagcagtctgagaagctcgagtggcccaagcactcgaacgaccttcctgtcatctcgtgggaggacttccaggccgagtccaagacccgtgcactcattgccgttcacggctttatccacgactgctcgtcgttcattgaggaccaccccggaggcgcccacctcattaagcgcgcgatcggcaccgactcgaccactgccttctttggtggtgtctacgaccactccaacgccgcccacaaccttctcgccatgatgcgcgtcggtgttcttgacggcggcatggaggtcgagcacctcaaggttggccgcctcacccgctccaactcggcagactcgctcgtctcggacgcgccttccagcgcatcctcgaccgtgtcggcgtcgtcgatcctctccgaggtcgaggacatggacaagcccgagcgcaagcccgtctaccagccggtcgcccaggtgtccaacccctggacgctcgccgtgcctccttcggagaagtatcgcatcatccgcacgtcccccgagatccgcccaggactcatctcgcgcatccagagcgccgcctcgcccagcctcacacgggcagcgagctttgacgctcctgtcgcgccttagagctttttctgttgagcacccgggtttccactaggcgccggtggttgtagcagtatatgcatcgttaatgggattgatcgtccgcggctatcgtcgaggttgtccaccgccgccctcagcttatcactcgctcgcttcatgtatgtgtatggcaactgtacggcaaagattgaagtgtcgagttccttttagtatcagatgtgacaaagtagagacgtcgagagcatctctgggccgcagcagcaagctcatctctcagtctccttcatgtcacgttatacattgccatctacagccaccttattattagagcatctcatcatgtactttatacaatgcattgcgcgtctcttgggtcaatgttcactttacaatgtcgtgacgtcgcacgcggtcgcctcctcctctcgcgtcagtacttctttcccttgcccttcccccagcgttcggcaacaaggacgcgcgaagcgccaactactgcctcgacgaggtcgcgcacgtcattagcggtgaccggaacaccatactgggccgacaaatggttggcaacggcagctagtggctcagggcgagccaacgcgaacaccgcaacctcgaaaacacgagccgcgtccgccgccggaatgtcgatgagcgcgcttccgcccacctgtgtcaaggtggggatgaacgtcgcccaccacactgcccgaagagcgtcctgtccgccctcagaacgaggaagggccttgatcgtagttaaaacgagtgtgtagctcgtttgtaagatccgggcaacgtggggtcgggctggcgtcggcccatctcgcatcagccgcgcaggaacatttactcaccgagtgcggcctccagagttgtgctctgatcgaaaatggcgtgcaagacgccgccaatgcctcccgcacgatcgccaacaatccgtttgacctcagctaaggtgaagtcaaggtgcattcccagggcggccgggaacgcaacaggtccgttggtcatcgtgcggtttaagtccgcggcgcgtcggacgatcgggcgataagagagcggcgtgcaatatcgcgtagcctcagacgcggccggcgtcagagagacacgcgaggttgcgcgc

SEQ ID NO: 13 - DNA, 5583 bp, Artificial Sequence
  Donor DNA including a knock in gene of interest (delta 12 desaturase coding sequence, aldo keto reductase promoter and terminator), selection marker (ura 5 gene -Orotate phosphoribosyltransferase-), and homology arms
aacagcaatcagacgcgtcttgcgggtgatggcctcggagccccaagcaaagttgcccgagtccagacggagggcgcggtacttggtgttgccgccacgggtgcgcacagtgtggatacgcttcgaagtgtcgagcttggtcatggccgactgacggccgagctcgaacttgcgcttcttgcggctgcctgtcagtatattgcaacgggaacatcgagttggtgcagggcagtaatgggacaagtgcgcagatttccctccctccgcttgcttgccggcagagcttcttctcccgaatccatcacaccgttccccgaatctgcacacttgaccccctgctagcccgcacaggcaagccactcactagtgggcgcggcgagcgccggatgcactgcgcttgtggcgggagtcacgagagatacccatttctgtcgttagtactaaaacgtgtgacaagtgccggagcacctccaggacaaggacagcggggcagacaggcttcgcggatggacaggatgcaggcgcagtcgccgaaagttcgtctggcgcatgtatttgccaagcgccgtcgaatgctgcagcggagtggtcgctggaaggatgccgaagatttgtcgatggggagggggatatgcgccgcgacaccgccgctgcggtcgcccaatgtgcgccctgtccatcgccgcttatgtcctgtgccgtcgctgtcgatgtcgaagggggtgctcggcgtgaggactcactgagttgtcggacgagaaacagaaggacccacgccgctgtagtcgacacaccttcgttaggcagactgtccaggaccaccatggctgtgaaccctgagctcgaggtcgtcggcgttaaagttgaggccgatcatgacagctcaactttcacgatttatcggggtcaaatgtatcatcccacgtcagctctggttggtgcctgattcaacccatctccgccggatagcgggccgagacgcaatccgcacttgagctcgttcatctctcctgcattactcacaatggctgctaccgacttcaaggccaactttattgagacggcgatcaacaccggggtcctcctcttcggcgagttcaccctcaagtctggccggtgagtaggtgcgacctgccgccgtcgtcgaatgtccaggctgacggccagcaagtccccgtacttcttcaacgccgggctcctgtacgacggcgctcttctctccgcgaccgccgacgcgtttgccggcacgctttccgcgatccccgagttcgatgtcctcttcggccccgcgtacaagggcatccccctcgcggccgtcacctgcgtcgctctcgcgaacaagggcatcaacaaggtctactgctacaaccgcaaggagaagaaggaccacggcgagggcggcacgctcgtcggcgcgcccatggcggacaagaaggtcgtgatcatcgacgacgttatgacggccggcacggcgattcgcgaagccatcgccattcttaaggagcagccgggcgcacagctcgttggtatcgtgcagctcgtcgaccgccaggagcgcggcaagggctcgacctcgaccagccaggaggtcgctgccgagtttggcgttccagttcttcccatcatctccatcggggacattatcacgtacctcaaggcccgtgggggatacgaggagcaggtcaaggctatcgaggcgtaccgcgccgagtacggcgttgtcgcctgaggcagctggtgtccgaggcgtcgaagccaagcgcggccgggatgtgaattgagcgggagataggatcccccatggtgccagatcttgggtaattgcgcgctgaaggccagattagagcatctcatcatgtactttatacaatgcattgcgcgtctcttggggtggagcagtaagcgttgtagatggtcgtcacaatcatagaggcgccctgcgcgtcccgcatgccgagtttgtaaaggtctctctcggtcgcatatgaacagctcaatccgctgcataaccaggaggcatgagaggggctggactactcatcgtcggggcagaagcgctgcgtgtccggacgaacttccggcatgtaggtggaccacacttcgggtgaaggggtgcgcctctgtgcgtatgagatgggacgcgcgcactttgcgagtttagagctttggacacttagacgacatgtcgaaggctctaaacgtacatccaccaacacagctaacagagggagtaagcggggctggactctcctcgttattatgagccgagaccccggcccggcggcagctcacggcagtcaggggcgtcggtagatgcccgggtgattcgacgtcaccacatttgggactatcaacacgacctcgtcagtgacagatgctggtgccccttccgacctcattatgcatggtagcgagggcgggacgaacgagcagtgctcgagcagcacatgtgcacattctcgctcgataaaaaagtgcaagtctgtcggcgtcatcccgacacgctcgcgacgaatgtccgcgtgtgtggtgtgctgctattccccgaaaacgccccgagggcaacatccgttcacccgcgctcacccagagcccacctgttctcacgccagccccaggccgcaggctgtataaagctcttccccgtccacttatctttcctcccattcttctctcccagtccaaacacaatgtctgccgccaccctgcgccagcgtaacgtcgacaagccaggtgctgccgacaaggccgagctcctccgtgaagccgaggacctcgagctcaccgagggccagaagtttgtcgtgcccaactttaccgtcaagcagctcttggacgccattccgtgagtgccctttgccccccccccatggcgcagaggcggatgtcggatggcttgcgtgagccacggcgtcggtggcaaacccatcactctaatcaatccgataagggacgcctgatggcggtgctcctcgcgtgccaactacggtgggccgcgggccgtcatggtgacgacgagacggacacaggacctcgttttgcgattccgtccgattaaactttacacccagaaccacgctcaccccagcgcccactgctacaagcgctcggcgttcaagtcgtcgctttacgtcctccaggactttgtcctcctcgccgccctcgtctacggcgcctaccacattgactccttcttgagccgcttgtgagtatttcccatcagatatcggtggagggaccgggaatccagcgacgcgggggtcgagtggagccatcatgtggctttttcatcccacctcgccgtgcctgcgtgccaagacaaggcaaccgtaggcacaatcgttgctccaccaccccaagtccccctcatggcagcatcatgctcggacttgctctcatgggtctctgatgcatgctcctgcggccagccgctaacatcgcagcaaccttggctcggttgcccacaccgccgccaagatcggcctctggttcacctaccaggtccttgccggcatggtcggtaccggtatctgggttatcgcccacgaatgcggccaccaggcctactccgagtccaagacgatcaacaacgccgtcggctgggtcctccactcgatccttcttgtgccttaccactcgtggcgcatctcgcacggccgtcaccacgccgccaccggccaccttacccgtgacgaggtctttgttccccgcacccgcgagcagctcggcatccaggcccccaagactgaggaggagaagaagggcatcaacgtccccgcttggcgccaggctgagcttcgtgaggccctcgaggagtcgcctatcggtgcgctctacggtgccatcctccaccagctcttcggctggcccatgtacctcatccgcaacgcgtccggccagctctggtaccccaagatgaccaaccacttccagccgtcgtcgatcatcttcaagccctcgcacttctggcagatcattgcttcggacattggtgttgttctcaccgccgccgccctcggcgtctttgtctactaccgtggctttgccgagatggctcgcatctacctcatcccctacctctgggtgaaccactggcttgtcttcatcaccttcctgcagcacaccgaccccgttctcccccactactcggagaagacttggacctttgcccgtggcgccctggcgaccattgaccgcaactgcctcggccccgtcggcccctacctcttccacggcatcaccgagacgcacgtcgcgcaccacacctcgtcgcgcatcccccactacaacgcgtgggaggcgaccgaggccctcaagaagttcctcggcccccactaccactacaaccccgagaacatgttcgtgtccttctggaaggcccaccgctactgcaagttcatcgaggcgggcgaagacgtcgccttctaccgcaacgccgctggtgtcgcgcagaaggtcggcatcatcgaggagaacggcgcggtgtccgactcgggcgtcgagcacaagtaagcgccggtggttgtagcagtatatgcatcgttaatgggattgatcgtccgcggctatcgtcgaggttgtccaccgccgccctcagcttatcactcgctcgcttcatgtatgtgtatggcaactgtacggcaaagattgaagtgtcgagttccttttagtatcagatgtgacaaagtagagacgtcgagagcatctctgggccgcagcagcaagctcatctctcagtctccttcatgtcacgttatacattgccatctacagccaccttattattagagcatctcatcatgtactttatacaatgcattgcgcgtctcttgggtcaatgttcactttacaatgtcgtgacgtcgcacgcggtcgcctcctcctctcgcgtcagtacttctttcccttgcccttcccccagcgttcggcaacaaggacgcgcgaagcgccaactactgcctcgacgaggtcgcgcacgtcattagcggtgaccggaacaccatactgggccgacaaatggttggcaacggcagctagtggctcagggcgagccaacgcgaacaccgcaacctcgaaaacacgagccgcgtccgccgccggaatgtcgatgagcgcgcttccgcccacctgtgtcaaggtggggatgaacgtcgcccaccacactgcccgaagagcgtcctgtccgccctcagaacgaggaagggccttgatcgtagttaaaacgagtgtgtagctcgtttgtaagatccgggcaacgtggggtcgggctggcgtcggcccatctcgcatcagccgcgcaggaacatttactcaccgagtgcggcctccagagttgtgctctgatcgaaaatggcgtgcaagacgccgccaatgcctcccgcacgatcgccaacaatccgtttgacctcagctaaggtgaagtcaaggtgcattcccagggcggccgggaacgcaacaggtccgttggtcatcgtgcggtttaagtccgcggcgcgtcggacgatcgggcgataagagagcggcgtgcaatatcgcgtagcctcagacgcggccggcgtcagagagacacgcgaggttgcgcgc

SEQ ID NO: 14 - RNA, 20 nt, Artificial Sequence
  crRNA sequence
gcaccaaccagagcugacgu

SEQ ID NO: 15 - RNA, 20 nt, Artificial Sequence
  crRNA sequence
ucuucccaucaucuccaucg

SEQ ID NO: 16 - RNA, 20 nt, Artificial Sequence
  crRNA sequence
gcuguagucgacacacccag

SEQ ID NO: 17 - RNA, 20 nt, Artificial Sequence
  crRNA sequence
gaacaccauacugggcgcug

SEQ ID NO: 18 - RNA, 20 nt, Artificial Sequence
  crRNA sequence
uggaugcucaucaagccucg

SEQ ID NO: 19 - RNA, 20 nt, Artificial Sequence
  crRNA sequence
uggacucggaguaggccugg

SEQ ID NO: 20 - RNA, 20 nt, Artificial Sequence
  crRNA sequence
aagaaacccaaguggcacau

SEQ ID NO: 21 - RNA, 20 nt, Artificial Sequence
  crRNA sequence
uguccgcuuccacaaagcag

SEQ ID NO: 22 - RNA, 20 nt, Artificial Sequence
  crRNA sequence
gugaccguaugaccguggca

SEQ ID NO: 23 - RNA, 20 nt, Artificial Sequence
  crRNA sequence
aggguggcggcagacauugu

SEQ ID NO: 24 - RNA, 20 nt, Artificial Sequence
  crRNA sequence
caacaugacuccaugaccca

SEQ ID NO: 25 - RNA, 20 nt, Artificial Sequence
  crRNA sequence
gacauugugggguggguuga

SEQ ID NO: 26 - RNA, 20 nt, Artificial Sequence
  crRNA sequence
cccauaaucaucaucaaguu

SEQ ID NO: 27 - DNA, 2699 bp, Artificial Sequence
  Donor DNA including the knock in gene of selection marker (ura 5 gene -Orotate phosphoribosyltransferase-), and homology arms for delta-12 desaturase knock out
ctttgccccccccccatggcgcagaggcggatgtcggatggcttgcgtgagccacggcgtcggtggcaaacccatcactctaatcaatccgataagggacgcctgatggcggtgctcctcgcgtgccaactacggtgggccgcgggccgtcatggtgacgacgagacggacacaggacctcgttttgcgattccgtccgattaaactttacacccagaaccacgctcaccccagcgcccctgctacaagcgctcggcgttcaagtcgtcgctttacgtcctccaggactttgtcctcctcgccgccctcgtctacggcgcctaccacattgactccttcttgagccgcttgtgagtatttcccatcagatatcggtggagggaccgggaatccagcgacgcgggggtcgagtggagccatcatgtggctttttcatcccacctcgccgtgcctgcgtgccaagacaaggcaaccgtaggcacaatcgttgctccaccaccccaagtccccctcatggcagcatcatgctcggacttgctctcatgggtctctgatgcatgctcctgcggccagccgctaacatcgcagcaaccttggctcggttgcccacaccgccgccaagatcggcctctggttcacctaccaggtccttgccggcatggtcggtaccggtatctgggttatcgcccacgaatgcggcgctggaaggatgccgaagatttgtcgatggggagggggatatgcgccgcgacaccgccgctgcggtcgcccaatgtgcgccctgtccatcgccgcttatgtcctgtgccgtcgctgtcgatgtcgaagggggtgctcggcgtgaggactcactgagttgtcggacgagaaacagaaggacccacgccgctgtagtcgacacacccagcggaggcagactgtccaggaccaccatggctgtgaaccctgagctcgaggtcgtcggcgttaaagttgaggccgatcatgacagctcaactttcacgatttatcggggtcaaatgtatcatcccacgtcagctctggttggtgcctgattcaacccatctccgccggatagcgggccgagacgcaatccgcacttgagctcgttcatctctcctgcattactcacaatggctgctaccgacttcaaggccaactttattgagacggcgatcaacaccggggtcctcctcttcggcgagttcaccctcaagtctggccggtgagtaggtgcgacctgccgccgtcgtcgaatgtccaggctgacggccagcaagtccccgtacttcttcaacgccgggctcctgtacgacggcgctcttctctccgcgaccgccgacgcgtttgccggcacgctttccgcgatccccgagttcgatgtcctcttcggccccgcgtacaagggcatccccctcgcggccgtcacctgcgtcgctctcgcgaacaagggcatcaacaaggtctactgctacaaccgcaaggagaagaaggaccacggcgagggcggcacgctcgtcggcgcgcccatggcggacaagaaggtcgtgatcatcgacgacgttatgacggccggcacggcgattcgcgaagccatcgccattcttaaggagcagccgggcgcacagctcgttggtatcgtgcagctcgtcgaccgccaggagcgcggcaagggctcgacctcgaccagccaggaggtcgctgccgagtttggcgttccagttcttcccatcatctccatcggggacattatcacgtacctcaaggcccgtgggggatacgaggagcaggtcaaggctatcgaggcgtaccgcgccgagtacggcgttgtcgcctgaggcagctggtgtccgaggcgtcgaagccaagcgcggccgggatgtgaattgagcgggagataggatcccccatggtgccagatcttgggtaattgcgcgctgaaggccagattagagcatctcatcatgtactttatacaatgcattgcgcgtctcttggggtcatactccgagtccaagacgatcaacaacgccgtcggctgggtcctccactcgatccttcttgtgccttaccactcgtggcgcatctcgcacggccgtcaccacgccgccaccggccaccttacccgtgacgaggtctttgttccccgcacccgcgagcagctcggcatccaggcccccaagactgaggaggagaagaagggcatcaacgtccccgcttggcgccaggctgagcttcgtgaggccctcgaggagtcgcctatcggtgcgctctacggtgccatcctccaccagctcttcggctggcccatgtacctcatccgcaacgcgtccggccagctctggtaccccaagatgaccaaccacttccagccgtcgtcgatcatcttcaagccctcgcacttctggcagatcattgcttcggacattggtgttgttctcaccgccgccgccctcggcgtctttgtctactaccgtggctttgccgagatggctcgcatctacctcatcccctacctctgggtgaaccactggcttgtcttcatcaccttcctgcagcacaccgaccccgttctcccccactactcggagaagacttggacctttgcccgtggcgccctggcgaccattgaccgcaactgcctcggccccgtcggcccctacctcttccacggcatcaccgagacgcacgtcgcgcac